European Patent Application EP 4 375 288 A1, published May 29, 2024. Title: POLYPEPTIDE TARGETING INTEGRIN ALPHA 6 AND USE THEREOF. Applicant: GUANGZHOU GENBIONOVA MEDICAL TECHNOLOGY CO., LTD. The sequence listing filed with the application follows.

SEQUENCE LISTING (18 sequences)

SEQ ID NO: 1 - protein, 4 aa, Artificial Sequence
  Synthesized
RWYD

SEQ ID NO: 2 - protein, 9 aa, Artificial Sequence
  Synthesized
CRWYDENAC

SEQ ID NO: 3 - protein, 9 aa, Artificial Sequence
  Synthesized
CAWYDENAC

SEQ ID NO: 4 - protein, 9 aa, Artificial Sequence
  Synthesized
CRAYDENAC

SEQ ID NO: 5 - protein, 9 aa, Artificial Sequence
  Synthesized
CRWADENAC

SEQ ID NO: 6 - protein, 9 aa, Artificial Sequence
  Synthesized
CRWYAENAC

SEQ ID NO: 7 - protein, 9 aa, Artificial Sequence
  Synthesized
CRWYDANAC

SEQ ID NO: 8 - protein, 9 aa, Artificial Sequence
  Synthesized
CRWYDEAAC

SEQ ID NO: 9 - protein, 7 aa, Artificial Sequence
  Synthesized
RWYDENA

SEQ ID NO: 10 - protein, 6 aa, Artificial Sequence
  Synthesized
RWYDEN

SEQ ID NO: 11 - protein, 7 aa, Artificial Sequence
  Synthesized
RWYDANA

SEQ ID NO: 12 - protein, 6 aa, Artificial Sequence
  Synthesized
RWYDAN

SEQ ID NO: 13 - protein, 6 aa, Artificial Sequence
  Synthesized
RWYDEA

SEQ ID NO: 14 - protein, 5 aa, Artificial Sequence
  Synthesized
RWYDE

SEQ ID NO: 15 - protein, 5 aa, Artificial Sequence
  Synthesized
RWYDA

SEQ ID NO: 16 - protein, 6 aa, Artificial Sequence
  Synthesized
RWYAEN

SEQ ID NO: 17 - protein, 5 aa, Artificial Sequence
  Synthesized
RWYAE

SEQ ID NO: 18 - protein, 3 aa, Artificial Sequence
  Synthesized
RWY